European Patent Application EP 4 239 065 A1, published September 6, 2023. Title: MUTANT CIS-PRENYLTRANSFERASE (CPT) FAMILY PROTEIN, METHOD FOR PRODUCING POLYISOPRENOID, VECTOR, TRANSGENIC PLANT, METHOD FOR PRODUCING PNEUMATIC TIRE, AND METHOD FOR PRODUCING RUBBER PRODUCT. Applicant: SUMITOMO RUBBER INDUSTRIES, LTD. Application EP. The sequence listing filed with the application follows.

SEQUENCE LISTING (34 sequences)

SEQ ID NO: 1 - protein, 290 aa, Hevea brasiliensis
MELYNGERPSVFRLLGKYMRKGLYSILTQGPIPTHIAFILDGNRRFAKKHKLPEGGGHKAGFLALLNVLTYCYELGVKYATIYAFSIDNFRRKPHEVQYVMDLMLEKIEGMIMEESIINAYDICVRFVGNLKLLSEPVKTAADKIMRATANNSKCVLLIAVCYTSTDEIVHAVEESSELNSNEVCNNQELEEANATGSGTVIQIENMESYSGIKLVDLEKNTYINPYPDVLIRTSGETRLSNYLLWQTTNCILYSPHALWPEIGLRHVVWAVINFQRHYSYLEKHKEYLK

SEQ ID NO: 2 - DNA, 873 bp, Hevea brasiliensis
  source 1..873: mol_type = genomic DNA
atggaattatacaacggtgagaggccaagtgtgttcagacttttagggaagtatatgagaaaagggttatatagcatcctaacccagggtcccatccctactcatattgccttcatattggatggaaacaggaggtttgctaagaagcataaactgccagaaggaggtggtcataaggctggatttttagctcttctgaacgtactaacttattgctatgagttaggagtgaaatatgcgactatctatgcctttagcatcgataattttcgaaggaaacctcatgaggttcagtacgtaatggatctaatgctggagaagattgaagggatgatcatggaagaaagtatcatcaatgcatatgatatttgcgtacgttttgtgggtaacctgaagcttttaagtgagccagtcaagaccgcagcagataagattatgagggctactgccaacaattccaaatgtgtgcttctcattgctgtatgctatacttcaactgatgagatcgtgcatgctgttgaagaatcctctgaattgaactccaatgaagtttgtaacaatcaagaattggaggaggcaaatgcaactggaagcggtactgtgattcaaattgagaacatggagtcgtattctggaataaaacttgtagaccttgagaaaaacacctacataaatccttatcctgatgttctgattcgaacttctggggagacccgtctgagcaactacttactttggcagactactaattgcatactgtattctcctcatgcactgtggccagagattggtcttcgacacgtggtgtgggcagtaattaacttccaacgtcattattcttacttggagaaacataaggaatacttaaaataa

SEQ ID NO: 3 - protein, 302 aa, Arabidopsis thaliana
MLSILSSLLSLLFLFIISCFFITSHFWFPLSLPKILGFIKITSSRDDYDNEQRDEGTYVVGVEELQRELMPRHVAVIMDGNRRWAKRAGLLTSQGHEAGAKRLIEFSELCFKLGIHTVSAFAFSTENWGRHKIEVKCLMSLIQHYLKSKIQYFQREETRVSVIGNLTKIPESLLRTVQEIEEATRSYKKKHLILAIDYSGRLDILRACKSIVKKSEKGLIREEDVDEALIERELLTNCTEFPSPDLLIRTSGEQRISNFFLWQLAYTELFFSPVLWPDFDKDKLLEALVSYQRRERRFGCRV

SEQ ID NO: 4 - protein, 368 aa, Hevea brasiliensis
MEIFEAGRPSVLASLGRFIRKCIFRILSIGPIPSHVAFIMDGNRRFAKKEKLEEGSGHRAGSLALMSTLKYCYELGVKYVTIYAFSIDNFRRRPDEVQLIMDLILEKIEGLLRDENVVNAYGIRVRFVGTLKLLSEPVRVAAEKVARASAKNTKFVLVICIAYSSTDEIVHAVQESCKYKLNKIEPSNSNRACNDANEQVEENGKKIDSTITHGVQESCKDETDKSRTINAKPMYNGVTKEAGGTDNANTVIVNSIGDKWDDAHELEATRTGNGVISVEEIDKMLSHSSIKLVDIEKKLHMAVAPDPDILVRTSGESRLSNFLLWQTSNCSLYSPKALWPEIGLRHLVWAVITFQRNHSYLEKKKKQL

SEQ ID NO: 5 - DNA, 909 bp, Arabidopsis thaliana
  source 1..909: mol_type = genomic DNA
atgttgtctattctctcttctcttttatctctcctttttctgtttatcatctcttgtttcttcatcacaagccatttttggttccctctttccttgccaaaaatactcggattcatcaaaatcacatcttcgagagacgattatgacaacgagcaacgtgacgagggaacttatgtggtaggagtggaggagctacaaagagagctgatgccaagacatgtggcagtgataatggacggaaaccggagatgggccaaacgggccggattgctgacgtcacaaggccacgaggccggagctaaacggcttatagagttctccgagctttgctttaaattggggattcatacagtttcagcttttgccttctccacagagaattggggaagacacaagattgaggttaagtgcttgatgtctttgatccaacattacctcaagtccaagatccaatatttccaaagagaggaaactcgagtttctgttatcgggaacctaacgaagatccctgagtctctcctccgaacagtccaagagatagaggaagctacgagaagctataagaagaagcatctcatattggcaatagattacagcgggagattagacatcttgcgagcttgcaagagtattgtgaagaaatcagaaaaagggttgatccgagaggaagatgtagacgaggcattgatcgaaagagagcttctgacaaattgtactgagttcccaagtcctgatctattgattaggacaagtggagaacagaggattagtaacttcttcttgtggcaacttgcttatacagagctcttcttctcgccggtcctttggcctgatttcgataaggataagcttctagaggccctggtttcgtatcagcgccgggaaagacgatttggctgtcgggtttga

SEQ ID NO: 6 - DNA, 1107 bp, Hevea brasiliensis
  source 1..1107: mol_type = genomic DNA
atggaaatatttgaggctggtaggccaagcgtgcttgcaagtttggggagatttatcagaaaatgcatatttcgcattctatcaataggtcccatcccaagtcatgttgccttcataatggatggaaaccggaggtttgctaagaaggagaaactggaagaaggatctggtcacagggctggatctttagctctaatgtccacgcttaagtactgctatgagttgggagtgaagtatgtgactatatatgccttcagcattgataattttagaaggcgacctgatgaggttcagctcataatggatctaatactggagaagattgaggggctgctcagggacgaaaatgttgtcaatgcatatggcatcagagtacgatttgtaggtaccttgaagcttctaagtgagccagtcagggtcgcagcagaaaaagtcgccagggctagtgccaagaataccaagtttgtgcttgtcatttgtatagcctattcttcaactgatgagattgtgcatgctgttcaagaatcttgtaaatataaattgaacaaaattgagccatctaactccaacagggcttgcaatgatgcgaatgaacaagtagaagaaaatggtaagaagatagatagtaccatcacacatggtgttcaagaatcctgcaaagatgaaacagataaatctcgcacaataaacgcaaagccaatgtataatggtgtgaccaaagaagctggagggactgacaatgctaatactgtgatagtaaattccatcggagacaagtgggatgatgctcacgaactggaggcaactagaactggcaatggtgtgatttcagtagaagaaattgataagatgctgtcacattctagcataaagctggtagacattgagaaaaaattgcacatggctgtagcccctgatcctgatatcttggttcgaacttctggagagagccgtctgagcaacttcctactttggcagactagtaactgttcactgtattctccaaaggcactgtggccggagattggcctacgccacttggtgtgggcagtaataaccttccaacgtaatcattcttatttggagaagaaaaagaagcagttgtaa

SEQ ID NO: 7 - protein, 268 aa, synthetic construct
MELYNGERPSVFRLLGKYMRKGLYSILTQGPIPTHVAVIMDGNRRWAKRAGLLTSQGHEAGAKRLIEFSELCFKLGIHTVSAFAFSTENWGRHKIEVKCLMSLIQHYLKSKIQYFQREETRVSVIGNLTKIPESLLRTVQEIEEATRSYKKKHLILAIDYSGRLDILRACKSIVKKSEKGLIREEDVDEALIERELLTNCTEFPSPDLLIRTSGEQRISNFFLWQLAYTELFFSPVLWPDIGLRHVVWAVINFQRHYSYLEKHKEYLK

SEQ ID NO: 8 - DNA, 807 bp, synthetic construct
  source 1..807: mol_type = other DNA
atggaattatacaacggtgagaggccaagtgtgttcagacttttagggaagtatatgagaaaagggttatatagcatcctaacccagggtcccatccctactcatgtggcagtgataatggacggaaaccggagatgggccaaacgggccggattgctgacgtcacaaggccacgaggccggagctaaacggcttatagagttctccgagctttgctttaaattggggattcatacagtttcagcttttgccttctccacagagaattggggaagacacaagattgaggttaagtgcttgatgtctttgatccaacattacctcaagtccaagatccaatatttccaaagagaggaaactcgagtttctgttatcgggaacctaacgaagatccctgagtctctcctccgaacagtccaagagatagaggaagctacgagaagctataagaagaagcatctcatattggcaatagattacagcgggagattagacatcttgcgagcttgcaagagtattgtgaagaaatcagaaaaagggttgatccgagaggaagatgtagacgaggcattgatcgaaagagagcttctgacaaattgtactgagttcccaagtcctgatctattgattaggacaagtggagaacagaggattagtaacttcttcttgtggcaacttgcttatacagagctcttcttctcgccggtcctttggcctgatattggtcttcgacacgtggtgtgggcagtaattaacttccaacgtcattattcttacttggagaaacataaggaatacttaaaataa

SEQ ID NO: 9 - DNA, 417 bp, Hevea brasiliensis
  source 1..417: mol_type = genomic DNA
atggctgaagacgaagacaaccaacaagggcagggggaggggttaaaatatttgggttttgtgcaagacgcggcaacttatgctgtgactaccttctcaaacgtctatctttttgccaaagacaaatctggtccactgcagcctggtgtcgatatcattgagggtccggtgaagaacgtggctgtacctctctataataggttcagttatattcccaatggagctctcaagtttgtagacagcacggttgttgcatctgtcactattatagatcgctctcttcccccaattgtcaaggacgcatctatccaagttgtttcagcaattcgagctgccccagaagctgctcgttctctggcttcttctttgcctgggcagaccaagatacttgctaaggtgttttatggagagaattga

SEQ ID NO: 10 - protein, 138 aa, Hevea brasiliensis
MAEDEDNQQGQGEGLKYLGFVQDAATYAVTTFSNVYLFAKDKSGPLQPGVDIIEGPVKNVAVPLYNRFSYIPNGALKFVDSTVVASVTIIDRSLPPIVKDASIQVVSAIRAAPEAARSLASSLPGQTKILAKVFYGEN

SEQ ID NO: 11 - DNA, 795 bp, synthetic construct
  source 1..795: mol_type = other DNA
atggaattatacaacggtgagaggccaagtgtgttcagacttttagggaagtatatgagaaaagggttatatagcatcctaacccagggtcccatccctactcatgtggcagtgataatggacggaaaccggagatgggccaaacgggccggattgctgacgtcacaaggccacgaggccggagctaaacggcttatagagttctccgagctttgctttaaattggggattcatacagtttcagcttttgccttctccacagagaattggggaagacacaagattgaggttaagtgcttgatgtctttgatccaacattacctcaagtccaagatccaatatttccaaagagaggaaactcgagtttctgttatcgggaacctaacgaagatccctgagtctctcctccgaacagtccaagagatagaggaagctacgagaagctataagaagaagcatctcatattggcaatagattacagcgggagattagacatcttgcgagcttgcaagagtattgtgaagaaatcagaaaaagggttgatccgagaggaagatgtagacgaggcattgatcgaaagagagcttctgacaaattgtactgagttcccaagtcctgatctattgattaggacaagtggagaacagaggattagtaacttcttcttgtggcaacttgcttatacagagctcttcttctcgccggtcctttggcctgatttcgataaggataagcttctagaggccctggtttcgtatcagcgccgggaaagacgatttggctgtcgggtttga

SEQ ID NO: 12 - protein, 264 aa, synthetic construct
MELYNGERPSVFRLLGKYMRKGLYSILTQGPIPTHVAVIMDGNRRWAKRAGLLTSQGHEAGAKRLIEFSELCFKLGIHTVSAFAFSTENWGRHKIEVKCLMSLIQHYLKSKIQYFQREETRVSVIGNLTKIPESLLRTVQEIEEATRSYKKKHLILAIDYSGRLDILRACKSIVKKSEKGLIREEDVDEALIERELLTNCTEFPSPDLLIRTSGEQRISNFFLWQLAYTELFFSPVLWPDFDKDKLLEALVSYQRRERRFGCRV

SEQ ID NO: 13 - DNA, 34 bp, synthetic construct
  misc_feature 1..34: note = PRIMER-1
  source 1..34: mol_type = other DNA
tttggatccgatggaattatacaacggtgagagg

SEQ ID NO: 14 - DNA, 39 bp, synthetic construct
  misc_feature 1..39: note = PRIMER-2
  source 1..39: mol_type = other DNA
tttgcggccgcttattttaagtattccttatgtttctcc

SEQ ID NO: 15 - DNA, 27 bp, synthetic construct
  misc_feature 1..27: note = PRIMER-3
  source 1..27: mol_type = other DNA
tttctcgagatggctgaagacgaagac

SEQ ID NO: 16 - DNA, 28 bp, synthetic construct
  misc_feature 1..28: note = PRIMER-4
  source 1..28: mol_type = other DNA
tttggatcctcaattctctccataaaac

SEQ ID NO: 17 - DNA, 25 bp, synthetic construct
  misc_feature 1..25: note = PRIMER-5
  source 1..25: mol_type = other DNA
tcccatccctactcatgtggcagtg

SEQ ID NO: 18 - DNA, 34 bp, synthetic construct
  misc_feature 1..34: note = PRIMER-6
  source 1..34: mol_type = other DNA
tacaggttttcctcgagtcaaacccgacagccaa

SEQ ID NO: 19 - DNA, 40 bp, synthetic construct
  misc_feature 1..40: note = PRIMER-7
  source 1..40: mol_type = other DNA
acatcaccaagatatcatggaattatacaacggtgagagg

SEQ ID NO: 20 - DNA, 25 bp, synthetic construct
  misc_feature 1..25: note = PRIMER-8
  source 1..25: mol_type = other DNA
cactgccacatgagtagggatggga

SEQ ID NO: 21 - DNA, 25 bp, synthetic construct
  misc_feature 1..25: note = PRIMER-9
  source 1..25: mol_type = other DNA
tcccatccctactcatgtggcagtg

SEQ ID NO: 22 - DNA, 26 bp, synthetic construct
  misc_feature 1..26: note = PRIMER-10
  source 1..26: mol_type = other DNA
gtcgaagaccaatatcaggccaaagg

SEQ ID NO: 23 - DNA, 26 bp, synthetic construct
  misc_feature 1..26: note = PRIMER-11
  source 1..26: mol_type = other DNA
cctttggcctgatattggtcttcgac

SEQ ID NO: 24 - DNA, 27 bp, synthetic construct
  misc_feature 1..27: note = PRIMER-12
  source 1..27: mol_type = other DNA
tacaggttttcctcgagttattttaag

SEQ ID NO: 25 - DNA, 40 bp, synthetic construct; identical to SEQ ID NO: 19
  misc_feature 1..40: note = PRIMER-13
  source 1..40: mol_type = other DNA

SEQ ID NO: 26 - DNA, 34 bp, synthetic construct; identical to SEQ ID NO: 18
  misc_feature 1..34: note = PRIMER-14
  source 1..34: mol_type = other DNA

SEQ ID NO: 27 - DNA, 40 bp, synthetic construct; identical to SEQ ID NO: 19
  misc_feature 1..40: note = PRIMER-15
  source 1..40: mol_type = other DNA

SEQ ID NO: 28 - DNA, 27 bp, synthetic construct
  misc_feature 1..27: note = PRIMER-16
  source 1..27: mol_type = other DNA
tacaggttttcctcgagttattttaag

SEQ ID NO: 29 - DNA, 46 bp, synthetic construct
  misc_feature 1..46: note = PRIMER-17
  source 1..46: mol_type = other DNA
acatcaccaagatatcatgttgtctattctctcttctcttttatct

SEQ ID NO: 30 - DNA, 35 bp, synthetic construct
  misc_feature 1..35: note = PRIMER-18
  source 1..35: mol_type = other DNA
tgattggccgaggcggcctcaaacccgacagccaa

SEQ ID NO: 31 - DNA, 40 bp, synthetic construct; identical to SEQ ID NO: 19
  misc_feature 1..40: note = PRIMER-19
  source 1..40: mol_type = other DNA

SEQ ID NO: 32 - DNA, 34 bp, synthetic construct; identical to SEQ ID NO: 18
  misc_feature 1..34: note = PRIMER-20
  source 1..34: mol_type = other DNA

SEQ ID NO: 33 - DNA, 40 bp, synthetic construct; identical to SEQ ID NO: 19
  misc_feature 1..40: note = PRIMER-21
  source 1..40: mol_type = other DNA

SEQ ID NO: 34 - DNA, 27 bp, synthetic construct
  misc_feature 1..27: note = PRIMER-22
  source 1..27: mol_type = other DNA
tacaggttttcctcgagttattttaag